European Patent Application EP 4 722 368 A1, published April 8, 2026. Title: A Novel Nucleic Acid Construct Comprising poly(A) Tail Having Secondary or Tertiary Structure and Uses Thereof. Applicant: Samsung Biologics Co. , Ltd. The sequence listing filed with the application follows.

SEQUENCE LISTING (119 sequences)

SEQ ID NO: 1 - RNA, 41 nt, synthetic construct
  source 1..41: mol_type = other RNA
agagagcagatctctgttgaataaccaacgtcaatatgctg

SEQ ID NO: 2 - RNA, 40 nt, synthetic construct
  source 1..40: mol_type = other RNA
gagagcagatctctgttgaataaccaacgtcaatatgctg

SEQ ID NO: 3 - RNA, 41 nt, synthetic construct
  source 1..41: mol_type = other RNA
atccggttgcgttgtgaatcgcgccactcctaacttggacc

SEQ ID NO: 4 - RNA, 41 nt, synthetic construct
  source 1..41: mol_type = other RNA
tccggttgcgttgtgaatcgcgcccacacctaacttggacc

SEQ ID NO: 5 - RNA, 41 nt, synthetic construct
  source 1..41: mol_type = other RNA
tccggttgcgttgtggttgaataaccaacctaacttggacc

SEQ ID NO: 6 - RNA, 41 nt, synthetic construct
  source 1..41: mol_type = other RNA
ccgtcgattgtccacgttgaataaccaaccggacgctagcc

SEQ ID NO: 7 - RNA, 28 nt, synthetic construct
  source 1..28: mol_type = other RNA
agagcagatgttgaataaccaacgtctg

SEQ ID NO: 8 - RNA, 31 nt, synthetic construct
  source 1..31: mol_type = other RNA
agagagcagatctgatacaacgtcaatgctg

SEQ ID NO: 9 - RNA, 27 nt, synthetic construct
  source 1..27: mol_type = other RNA
agagagcagatctctgtcaatatgctg

SEQ ID NO: 10 - RNA, 40 nt, synthetic construct
  source 1..40: mol_type = other RNA
cagcatattgacgctgggaaagaccagagatctgctctct

SEQ ID NO: 11 - RNA, 40 nt, synthetic construct
  source 1..40: mol_type = other RNA
ggtccaagttaggaaagtatcaactcgcaacgcaaccgga

SEQ ID NO: 12 - RNA, 40 nt, synthetic construct
  source 1..40: mol_type = other RNA
cagcatattgacttggttattcaacagagatctgctctct

SEQ ID NO: 13 - RNA, 40 nt, synthetic construct
  source 1..40: mol_type = other RNA
ggtccaagttaggcgtgtatcaactcgcaacgcaaccgga

SEQ ID NO: 14 - RNA, 40 nt, synthetic construct
  source 1..40: mol_type = other RNA
ggtccaagttaggctgggaaagacccgcaacgcaaccgga

SEQ ID NO: 15 - RNA, 40 nt, synthetic construct
  source 1..40: mol_type = other RNA
ggctagcgtccggctgggaaagaccgtggacaatcgacgg

SEQ ID NO: 16 - RNA, 27 nt, synthetic construct
  source 1..27: mol_type = other RNA
cagacgctgggaaagaccatctgctct

SEQ ID NO: 17 - RNA, 30 nt, synthetic construct
  source 1..30: mol_type = other RNA
cagcattgacgctggagagatctgctctct

SEQ ID NO: 18 - RNA, 27 nt, synthetic construct
  source 1..27: mol_type = other RNA
cagcatattgacagagatctgctctct

SEQ ID NO: 19 - RNA, 42 nt, synthetic construct
  source 1..42: mol_type = other RNA
ggcgctgcctacggaggtggcagccatctccttctcggcatc

SEQ ID NO: 20 - RNA, 44 nt, synthetic construct
  source 1..44: mol_type = other RNA
gcccgatgggcctcccaacgggccctcctcccctccttgcaccg

SEQ ID NO: 21 - RNA, 1579 nt, synthetic construct
  source 1..1579: mol_type = other RNA
attgcttgcttgcttgcttgcttgcttgcttgggccttgaggcttacagcttcttcccttgggcattcattcccagttttgaggaggagaacccggacttttctggaaccgcgaggcagccgaggccctgggtgccgccaagaagctgcagcctgcacagacagccgccaagaacctcatcatcttcctgggcgatgggatgggggtgtctacggtgacagctgccaggatcctaaaagggcagaagaaggacaaactggggcctgagatacccctggccatggaccgcttcccatatgtggctctgtccaagacatacaatgtagacaaacatgtgccagacagtggagccacagccacggcctacctgtgcggggtcaagggcaacttccagaccattggcttgagtgcagccgcccgctttaaccagtgcaacacgacacgcggcaacgaggtcatctccgtgatgaatcgggccaagaaagcagggaagtcagtgggagtggtaaccaccacacgagtgcagcacgcctcgccagccggcacctacgcccacacggtgaaccgcaactggtactcggacgccgacgtgcctgcctcggcccgccaggaggggtgccaggacatcgctacgcagctcatctccaacatggacattgacgtgatcctaggtggaggccgaaagtacatgtttcgcatgggaaccccagaccctgagtacccagatgactacagccaaggtgggaccaggctggacgggaagaatctggtgcaggaatggctggcgaagcgccagggtgcccggtatgtgtggaaccgcactgagctcatgcaggcttccctggacccgtctgtgacccatctcatgggtctctttgagcctggagacatgaaatacgagatccaccgagactccacactggacccctccctgatggagatgacagaggctgccctgcgcctgctgagcaggaacccccgcggcttcttcctcttcgtggagggtggtcgcatcgaccatggtcatcatgaaagcagggcttaccgggcactgactgagacgatcatgttcgacgacgccattgagagggcgggccagctcaccagcgaggaggacacgctgagcctcgtcactgccgaccactcccacgtcttctccttcggaggctaccccctgcgagggagctccatcttcgggctggcccctggcaaggcccgggacaggaaggcctacacggtcctcctatacggaaacggtccaggctatgtgctcaaggacggcgcccggccggatgttaccgagagcgagagcgggagccccgagtatcggcagcagtcagcagtgcccctggacgaagagacccacgcaggcgaggacgtggcggtgttcgcgcgcggcccgcaggcgcacctggttcacggcgtgcaggagcagaccttcatagcgcacgtcatggccttcgccgcctgcctggagccctacaccgcctgcgacctggcgccccccgccggcaccaccgacgccgcgcacccgggttactctagagtcggggcggccggccgcttcgagcagacatga

SEQ ID NO: 22 - RNA, 558 nt, synthetic construct
  source 1..558: mol_type = other RNA
atgggagtcaaagttctgtttgccctgatctgcatcgctgtggccgaggccaagcccaccgagaacaacgaagacttcaacatcgtggccgtggccagcaacttcgcgaccacggatctcgatgctgaccgcgggaagttgcccggcaagaagctgccgctggaggtgctcaaagagatggaagccaatgcccggaaagctggctgcaccaggggctgtctgatctgcctgtcccacatcaagtgcacgcccaagatgaagaagttcatcccaggacgctgccacacctacgaaggcgacaaagagtccgcacagggcggcataggcgaggcgatcgtcgacattcctgagattcctgggttcaaggacttggagcccatggagcagttcatcgcacaggtcgatctgtgtgtggactgcacaactggctgcctcaaagggcttgccaacgtgcagtgttctgacctgctcaagaagtggctgccgcaacgctgtgcgacctttgccagcaagatccagggccaggtggacaagatcaagggggccggtggtgactaa

SEQ ID NO: 23 - RNA, 64 nt, synthetic construct
  source 1..64: mol_type = other RNA
aaaaaaaaaaaaaaaaaaaaaaaaaaaaaaaaaaaaaaaaaaaaaaaaaaaaaaaaaaaaaaaa

SEQ ID NO: 24 - RNA, 144 nt, synthetic construct
  source 1..144: mol_type = other RNA
aaaaaaaaaaaaaaaaaaaaaaaaaaaaaaaagagagcagatctctgttgaataaccaacgtcaatatgctgaaaaaaaaaaaaaaaaaaaaaaaaaaaaaaaacagcatattgacgctgggaaagaccagagatctgctctct

SEQ ID NO: 25 - RNA, 104 nt, synthetic construct
  source 1..104: mol_type = other RNA
aaaaaaaaaaaaaaaaaaaaaaaaaaaaaaaagagagcagatctctgttgaataaccaacgtcaatatgctgaaaaaaaaaaaaaaaaaaaaaaaaaaaaaaaa

SEQ ID NO: 26 - RNA, 144 nt, synthetic construct
  source 1..144: mol_type = other RNA
aaaaaaaaaaaaaaaaaaaaaaaaaaaaaaaagagagcagatctctgttgaataaccaacgtcaatatgctgaaaaaaaaaaaaaaaaaaaaaaaaaaaaaaaaagagagcagatctctggtctttcccagcgtcaatatgctg

SEQ ID NO: 27 - RNA, 79 nt, synthetic construct
  source 1..79: mol_type = other RNA
aaaaaaaaaaaaaaaaaaaaaaaaaaaaaaaaaaaaaaaaaaaaaaaaaaaaaaaaaaaaaaaaaaaaaaaaaaaaaaa

SEQ ID NO: 28 - RNA, 100 nt, synthetic construct
  source 1..100: mol_type = other RNA
aaaaaaaaaaaaaaaaaaaaaaaaaaaaaaaaaaaaaaaaaaaaaaaaaaaaaaaaaaaaaaaaaaaaaaaaaaaaaaaaaaaaaaaaaaaaaaaaaaaa

SEQ ID NO: 29 - RNA, 181 nt, synthetic construct
  source 1..181: mol_type = other RNA
aaaaaaaaaaaaaaaaaaaaaaaaaaaaaaaaaaaaaaaaaaaaaaaaaaagagagcagatctctgttgaataaccaacgtcaatatgctgaaaaaaaaaaaaaaaaaaaaaaaaaaaaaaaaaaaaaaaaaaaaaaaaaacagcatattgacgctgggaaagaccagagatctgctctct

SEQ ID NO: 30 - RNA, 161 nt, synthetic construct
  source 1..161: mol_type = other RNA
aaaaaaaaaaaaaaaaaaaaaaaaaaaaaaaaaaaaaaaaaaaaaaaaagagagcagatctctgttgaataaccaacgtcaatatgctgaaaaaaaaaaaaaaaaaaaaaaaaaaaaaaaacagcatattgacgctgggaaagaccagagatctgctctct

SEQ ID NO: 31 - RNA, 161 nt, synthetic construct
  source 1..161: mol_type = other RNA
aaaaaaaaaaaaaaaaaaaaaaaaaaaaaaaaagagagcagatctctgttgaataaccaacgtcaatatgctgaaaaaaaaaaaaaaaaaaaaaaaaaaaaaaaaaaaaaaaaaaaaaaaacagcatattgacgctgggaaagaccagagatctgctctct

SEQ ID NO: 32 - RNA, 159 nt, synthetic construct
  source 1..159: mol_type = other RNA
aaaaaaaaaaaaaaaaaaaaaaaaaaaaaaaaaaaaaaaaaaaaaaagagagcagatctctgttgaataaccaacgtcaatatgctgaaaaaaaaaaaaaaaaaaaaaaaaaaaaaaaacagcatattgacgctgggaaagaccagagatctgctctct

SEQ ID NO: 33 - RNA, 139 nt, synthetic construct
  source 1..139: mol_type = other RNA
aaaaaaaaaaaaaaaaaaaaaaaaaaaaaaaaaaaaaaaaaaaaaaagagagcagatctctgttgaataaccaacgtcaatatgctgaaaaaaaaaaaacagcatattgacgctgggaaagaccagagatctgctctct

SEQ ID NO: 34 - RNA, 144 nt, synthetic construct
  source 1..144: mol_type = other RNA
aaaaaaaaaaaaaaaaaaaaaaaaaaaaaaaaaaaaaaaaaagagagcagatctctgttgaataaccaacgtcaatatgctgaaaaaaaaaaaaaaaaaaaaaacagcatattgacgctgggaaagaccagagatctgctctct

SEQ ID NO: 35 - RNA, 144 nt, synthetic construct
  source 1..144: mol_type = other RNA
aaaaaaaaaaaaaaaaaaaaaaaaaaaaaaaaaaaaaaaaaaaaaaaaaaaagagagcagatctctgttgaataaccaacgtcaatatgctgaaaaaaaaaaaacagcatattgacgctgggaaagaccagagatctgctctct

SEQ ID NO: 36 - RNA, 159 nt, synthetic construct
  source 1..159: mol_type = other RNA
aaaaaaaaaaaaaaaaaaaaaaaaaaaaaaaaaaaaaaaaaaaaaaaaaaaaaaaaagagagcagatctctgttgaataaccaacgtcaatatgctgaaaaaaaaaaaaaaaaaaaaaacagcatattgacgctgggaaagaccagagatctgctctct

SEQ ID NO: 37 - RNA, 159 nt, synthetic construct
  source 1..159: mol_type = other RNA
aaaaaaaaaaaaaaaaaaaaaaaaaaaaaaaaaaaaaaaaaaaaaaaaaaaaaaaaaaaaaaaaaaagagagcagatctctgttgaataaccaacgtcaatatgctgaaaaaaaaaaaacagcatattgacgctgggaaagaccagagatctgctctct

SEQ ID NO: 38 - RNA, 159 nt, synthetic construct
  source 1..159: mol_type = other RNA
aaaaaaaaaaaaaaaaaaaaaaaaaaaaaaaaaaaaaaaaaaaaaaaaaaaaaaaaaaaaaaagagagcagatctctgttgaataaccaacgtcaatatgctgaaaaaaaaaaaaaaaacagcatattgacgctgggaaagaccagagatctgctctct

SEQ ID NO: 39 - RNA, 159 nt, synthetic construct
  source 1..159: mol_type = other RNA
aaaaaaaaaaaaaaaaaaaaaaaaaaaaaaaaaaaaaaaaaaaaaaaaaaaaaagagagcagatctctgttgaataaccaacgtcaatatgctgaaaaaaaaaaaaaaaaaaaaaaaaacagcatattgacgctgggaaagaccagagatctgctctct

SEQ ID NO: 40 - RNA, 151 nt, synthetic construct
  source 1..151: mol_type = other RNA
aaaaaaaaaaaaaaaaaaaaaaaaaaaaaaaaaaaaaaaaaaaaaaaaagagagcagatctctgttgaataaccaacgtcaatatgctgaaaaaaaaaaaaaaaaaaaaaacagcatattgacgctgggaaagaccagagatctgctctct

SEQ ID NO: 41 - RNA, 153 nt, synthetic construct
  source 1..153: mol_type = other RNA
aaaaaaaaaaaaaaaaaaaaaaaaaaaaaaaaaaaaaaaaaaaaaaaaagagagcagatctctgttgaataaccaacgtcaatatgctgaaaaaaaaaaaaaaaaaaaaaaaacagcatattgacgctgggaaagaccagagatctgctctct

SEQ ID NO: 42 - RNA, 155 nt, synthetic construct
  source 1..155: mol_type = other RNA
aaaaaaaaaaaaaaaaaaaaaaaaaaaaaaaaaaaaaaaaaaaaaaaaagagagcagatctctgttgaataaccaacgtcaatatgctgaaaaaaaaaaaaaaaaaaaaaaaaaacagcatattgacgctgggaaagaccagagatctgctctct

SEQ ID NO: 43 - RNA, 157 nt, synthetic construct
  source 1..157: mol_type = other RNA
aaaaaaaaaaaaaaaaaaaaaaaaaaaaaaaaaaaaaaaaaaaaaaaaagagagcagatctctgttgaataaccaacgtcaatatgctgaaaaaaaaaaaaaaaaaaaaaaaaaaaacagcatattgacgctgggaaagaccagagatctgctctct

SEQ ID NO: 44 - RNA, 159 nt, synthetic construct
  source 1..159: mol_type = other RNA
aaaaaaaaaaaaaaaaaaaaaaaaaaaaaaaaaaaaaaaaaaaaaaaaagagagcagatctctgttgaataaccaacgtcaatatgctgaaaaaaaaaaaaaaaaaaaaaaaaaaaaaacagcatattgacgctgggaaagaccagagatctgctctct

SEQ ID NO: 45 - RNA, 167 nt, synthetic construct
  source 1..167: mol_type = other RNA
aaaaaaaaaaaaaaaaaaaaaaaaaaaaaaaaaaaaaaaaaaaaaaaaagagagcagatctctgttgaataaccaacgtcaatatgctgaaaaaaaaaaaaaaaaaaaaaaaaaaaaaaaaaaaaaacagcatattgacgctgggaaagaccagagatctgctctct

SEQ ID NO: 46 - RNA, 169 nt, synthetic construct
  source 1..169: mol_type = other RNA
aaaaaaaaaaaaaaaaaaaaaaaaaaaaaaaaaaaaaaaaaaaaaaaaagagagcagatctctgttgaataaccaacgtcaatatgctgaaaaaaaaaaaaaaaaaaaaaaaaaaaaaaaaaaaaaaaacagcatattgacgctgggaaagaccagagatctgctctct

SEQ ID NO: 47 - RNA, 171 nt, synthetic construct
  source 1..171: mol_type = other RNA
aaaaaaaaaaaaaaaaaaaaaaaaaaaaaaaaaaaaaaaaaaaaaaaaagagagcagatctctgttgaataaccaacgtcaatatgctgaaaaaaaaaaaaaaaaaaaaaaaaaaaaaaaaaaaaaaaaaacagcatattgacgctgggaaagaccagagatctgctctct

SEQ ID NO: 48 - RNA, 163 nt, synthetic construct
  source 1..163: mol_type = other RNA
aaaaaaaaaaaaaaaaaaaaaaaaaaaaaaaaaaaaaaaaaaaaaaaaaaagagagcagatctctgttgaataaccaacgtcaatatgctgaaaaaaaaaaaaaaaaaaaaaaaaaaaaaaaacagcatattgacgctgggaaagaccagagatctgctctct

SEQ ID NO: 49 - RNA, 165 nt, synthetic construct
  source 1..165: mol_type = other RNA
aaaaaaaaaaaaaaaaaaaaaaaaaaaaaaaaaaaaaaaaaaaaaaaaaaaaagagagcagatctctgttgaataaccaacgtcaatatgctgaaaaaaaaaaaaaaaaaaaaaaaaaaaaaaaacagcatattgacgctgggaaagaccagagatctgctctct

SEQ ID NO: 50 - RNA, 169 nt, synthetic construct
  source 1..169: mol_type = other RNA
aaaaaaaaaaaaaaaaaaaaaaaaaaaaaaaaaaaaaaaaaaaaaaaaaaaaaaaaagagagcagatctctgttgaataaccaacgtcaatatgctgaaaaaaaaaaaaaaaaaaaaaaaaaaaaaaaacagcatattgacgctgggaaagaccagagatctgctctct

SEQ ID NO: 51 - RNA, 170 nt, synthetic construct
  source 1..170: mol_type = other RNA
aaaaaaaaaaaaaaaaaaaaaaaaaaaaaaaaaaaaaaaaaaaaaaaaaaaaaaaaaagagagcagatctctgttgaataaccaacgtcaatatgctgaaaaaaaaaaaaaaaaaaaaaaaaaaaaaaaacagcatattgacgctgggaaagaccagagatctgctctct

SEQ ID NO: 52 - RNA, 172 nt, synthetic construct
  source 1..172: mol_type = other RNA
aaaaaaaaaaaaaaaaaaaaaaaaaaaaaaaaaaaaaaaaaaaaaaaaaaaaaaaaaaaagagagcagatctctgttgaataaccaacgtcaatatgctgaaaaaaaaaaaaaaaaaaaaaaaaaaaaaaaacagcatattgacgctgggaaagaccagagatctgctctct

SEQ ID NO: 53 - RNA, 174 nt, synthetic construct
  source 1..174: mol_type = other RNA
aaaaaaaaaaaaaaaaaaaaaaaaaaaaaaaaaaaaaaaaaaaaaaaaaaaaaaaaaaaaaagagagcagatctctgttgaataaccaacgtcaatatgctgaaaaaaaaaaaaaaaaaaaaaaaaaaaaaaaacagcatattgacgctgggaaagaccagagatctgctctct

SEQ ID NO: 54 - RNA, 177 nt, synthetic construct
  source 1..177: mol_type = other RNA
aaaaaaaaaaaaaaaaaaaaaaaaaaaaaaaaaaaaaaaaaaaaaaaaaaaaaaaaaaaaaaaaagagagcagatctctgttgaataaccaacgtcaatatgctgaaaaaaaaaaaaaaaaaaaaaaaaaaaaaaaacagcatattgacgctgggaaagaccagagatctgctctct

SEQ ID NO: 55 - RNA, 179 nt, synthetic construct
  source 1..179: mol_type = other RNA
aaaaaaaaaaaaaaaaaaaaaaaaaaaaaaaaaaaaaaaaaaaaaaaaaaaaaaaaaaaaaaaaaaagagagcagatctctgttgaataaccaacgtcaatatgctgaaaaaaaaaaaaaaaaaaaaaaaaaaaaaaaacagcatattgacgctgggaaagaccagagatctgctctct

SEQ ID NO: 56 - RNA, 181 nt, synthetic construct
  source 1..181: mol_type = other RNA
aaaaaaaaaaaaaaaaaaaaaaaaaaaaaaaaaaaaaaaaaaaaaaaaaaaaaaaaaaaaaaaaaaaaagagagcagatctctgttgaataaccaacgtcaatatgctgaaaaaaaaaaaaaaaaaaaaaaaaaaaaaaaacagcatattgacgctgggaaagaccagagatctgctctct

SEQ ID NO: 57 - RNA, 183 nt, synthetic construct
  source 1..183: mol_type = other RNA
aaaaaaaaaaaaaaaaaaaaaaaaaaaaaaaaaaaaaaaaaaaaaaaaaaaaaaaaaaaaaaaaaaaaaaagagagcagatctctgttgaataaccaacgtcaatatgctgaaaaaaaaaaaaaaaaaaaaaaaaaaaaaaaacagcatattgacgctgggaaagaccagagatctgctctct

SEQ ID NO: 58 - RNA, 185 nt, synthetic construct
  source 1..185: mol_type = other RNA
aaaaaaaaaaaaaaaaaaaaaaaaaaaaaaaaaaaaaaaaaaaaaaaaaaaaaaaaaaaaaaaaaaaaaaaaagagagcagatctctgttgaataaccaacgtcaatatgctgaaaaaaaaaaaaaaaaaaaaaaaaaaaaaaaacagcatattgacgctgggaaagaccagagatctgctctct

SEQ ID NO: 59 - RNA, 187 nt, synthetic construct
  source 1..187: mol_type = other RNA
aaaaaaaaaaaaaaaaaaaaaaaaaaaaaaaaaaaaaaaaaaaaaaaaaaaaaaaaaaaaaaaaaaaaaaaaaaagagagcagatctctgttgaataaccaacgtcaatatgctgaaaaaaaaaaaaaaaaaaaaaaaaaaaaaaaacagcatattgacgctgggaaagaccagagatctgctctct

SEQ ID NO: 60 - RNA, 189 nt, synthetic construct
  source 1..189: mol_type = other RNA
aaaaaaaaaaaaaaaaaaaaaaaaaaaaaaaaaaaaaaaaaaaaaaaaaaaaaaaaaaaaaaaaaaaaaaaaaaaaagagagcagatctctgttgaataaccaacgtcaatatgctgaaaaaaaaaaaaaaaaaaaaaaaaaaaaaaaacagcatattgacgctgggaaagaccagagatctgctctct

SEQ ID NO: 61 - RNA, 191 nt, synthetic construct
  source 1..191: mol_type = other RNA
aaaaaaaaaaaaaaaaaaaaaaaaaaaaaaaaaaaaaaaaaaaaaaaaaaaaaaaaaaaaaaaaaaaaaaaaaaaaaaagagagcagatctctgttgaataaccaacgtcaatatgctgaaaaaaaaaaaaaaaaaaaaaaaaaaaaaaaacagcatattgacgctgggaaagaccagagatctgctctct

SEQ ID NO: 62 - RNA, 193 nt, synthetic construct
  source 1..193: mol_type = other RNA
aaaaaaaaaaaaaaaaaaaaaaaaaaaaaaaaaaaaaaaaaaaaaaaaaaaaaaaaaaaaaaaaaaaaaaaaaaaaaaaaagagagcagatctctgttgaataaccaacgtcaatatgctgaaaaaaaaaaaaaaaaaaaaaaaaaaaaaaaacagcatattgacgctgggaaagaccagagatctgctctct

SEQ ID NO: 63 - RNA, 197 nt, synthetic construct
  source 1..197: mol_type = other RNA
aaaaaaaaaaaaaaaaaaaaaaaaaaaaaaaaaaaaaaaaaaaaaaaaaaaaaaaaaaaaaaaaaaaaaaaaaaaaaaaaaaaaagagagcagatctctgttgaataaccaacgtcaatatgctgaaaaaaaaaaaaaaaaaaaaaaaaaaaaaaaacagcatattgacgctgggaaagaccagagatctgctctct

SEQ ID NO: 64 - RNA, 203 nt, synthetic construct
  source 1..203: mol_type = other RNA
aaaaaaaaaaaaaaaaaaaaaaaaaaaaaaaaaaaaaaaaaaaaaaaaaaaaaaaaaaaaaaaaaaaaaaaaaaaaaaaaaaaaaaaaaaagagagcagatctctgttgaataaccaacgtcaatatgctgaaaaaaaaaaaaaaaaaaaaaaaaaaaaaaaacagcatattgacgctgggaaagaccagagatctgctctct

SEQ ID NO: 65 - RNA, 209 nt, synthetic construct
  source 1..209: mol_type = other RNA
aaaaaaaaaaaaaaaaaaaaaaaaaaaaaaaaaaaaaaaaaaaaaaaaaaaaaaaaaaaaaaaaaaaaaaaaaaaaaaaaaaaaaaaaaaaaaaaaagagagcagatctctgttgaataaccaacgtcaatatgctgaaaaaaaaaaaaaaaaaaaaaaaaaaaaaaaacagcatattgacgctgggaaagaccagagatctgctctct

SEQ ID NO: 66 - RNA, 177 nt, synthetic construct
  source 1..177: mol_type = other RNA
aaaaaaaaaaaaaaaaaaaaaaaaaaaaaaaaaaaaaaaaaaaaaaaaagagagcagatctctgttgaataaccaacgtcaatatgctgaaaaaaaaaaaaaaaaaaaaaaaacagcatattgacgctgggaaagaccagagatctgctctctaaaaaaaaaaaaaaaaaaaaaaaa

SEQ ID NO: 67 - RNA, 168 nt, synthetic construct
  source 1..168: mol_type = other RNA
aaaaaaaaaaaaaaaaaaaaaaaaaaaaaaaagagagcagatctctgttgaataaccaacgtcaatatgctgaaaaaaaaaaaaaaaaaaaaaaaaaaaaaaaacagcatattgacgctgggaaagaccagagatctgctctctaaaaaaaaaaaaaaaaaaaaaaaa

SEQ ID NO: 68 - RNA, 183 nt, synthetic construct
  source 1..183: mol_type = other RNA
aaaaaaaaaaaaaaaaaaaaaaaaaaaaaaaaaaaaaaaaaaaaaaaaaaaaaaaaagagagcagatctctgttgaataaccaacgtcaatatgctgaaaaaaaaaaaaaaaaaaaaaacagcatattgacgctgggaaagaccagagatctgctctctaaaaaaaaaaaaaaaaaaaaaaaa

SEQ ID NO: 69 - RNA, 164 nt, synthetic construct
  source 1..164: mol_type = other RNA
aaaaaaaaaaaagaaaaaaaaaaaagaaaaaaaaaaaagaaaaaaaaaaaagaaaaaaaaagagagcagatctctgttgaataaccaacgtcaatatgctgaaaaaaaaaaaaaaaaaaaaaagcagcatattgacgctgggaaagaccagagatctgctctct

SEQ ID NO: 70 - RNA, 168 nt, synthetic construct
  source 1..168: mol_type = other RNA
aaaaaaaaaaaagaaaaaaaaaaaagaaaaaaaaaaaagaaaaaaaaaaaagaaaaaaaaaaaaggagagcagatctctgttgaataaccaacgtcaatatgctgaaaaaaaaaaaaaaaaaaaaaagcagcatattgacgctgggaaagaccagagatctgctctct

SEQ ID NO: 71 - RNA, 146 nt, synthetic construct
  source 1..146: mol_type = other RNA
aaaaaaaaaaaagaaaaaaaaaaaagaaaaaaaagagagcagatctctgttgaataaccaacgtcaatatgctgaaaaaaaaaaaaaaaaaaaaaaaaaaaaaaaacagcatattgacgctgggaaagaccagagatctgctctct

SEQ ID NO: 72 - RNA, 152 nt, synthetic construct
  source 1..152: mol_type = other RNA
aaaaaaaaaaaagaaaaaaaaaaaagaaaaaaaaaaaagagagagcagatctctgttgaataaccaacgtcaatatgctgaaaaaaaaaaaaaaaaaaaaaaaaaaaaaaaacagcatattgacgctgggaaagaccagagatctgctctct

SEQ ID NO: 73 - RNA, 156 nt, synthetic construct
  source 1..156: mol_type = other RNA
aaaaaaaaaaaagaaaaaaaaaaaagaaaaaaaaaaaagaaaaaaaaaaaaagagagcagatctctgttgaataaccaacgtcaatatgctgaaaaaaaaaaaaaaaaaaaaaaaacagcatattgacgctgggaaagaccagagatctgctctct

SEQ ID NO: 74 - RNA, 157 nt, synthetic construct
  source 1..157: mol_type = other RNA
aaaaaaaaaaaagaaaaaaaaaaaagaaaaaaaaaaaagaaaaaaaaaaaagagagagcagatctctgttgaataaccaacgtcaatatgctgaaaaaaaaaaaaaaaaaaaaaaaacagcatattgacgctgggaaagaccagagatctgctctct

SEQ ID NO: 75 - RNA, 161 nt, synthetic construct
  source 1..161: mol_type = other RNA
aaaaaaaaaaaaaaaaaaaaaaaaaaaaaaaaaaaaaaaaaaaaaaaaaaaaaaaaagagagcagatctctgttgaataaccaacgtcaatatgctgaaaaaaaaaaaagaaaaaaaaaagcagcatattgacgctgggaaagaccagagatctgctctct

SEQ ID NO: 76 - RNA, 163 nt, synthetic construct
  source 1..163: mol_type = other RNA
aaaaaaaaaaaaaaaaaaaaaaaaaaaaaaaaaaaaaaaaaaaaaaaaaaaaaaaaagagagcagatctctgttgaataaccaacgtcaatatgctgaaaaaaaaaaaagaaaaaaaaaaaagcagcatattgacgctgggaaagaccagagatctgctctct

SEQ ID NO: 77 - RNA, 146 nt, synthetic construct
  source 1..146: mol_type = other RNA
aaaaaaaaaaaaaaaaaaaaaaaaaaaaaaaagagagcagatctctgttgaataaccaacgtcaatatgctgaaaaaaaaaaaagaaaaaaaaaaaagaaaaaaaacagcatattgacgctgggaaagaccagagatctgctctct

SEQ ID NO: 78 - RNA, 151 nt, synthetic construct
  source 1..151: mol_type = other RNA
aaaaaaaaaaaaaaaaaaaaaaaaaaaaaaaagagagcagatctctgttgaataaccaacgtcaatatgctgaaaaaaaaaaaagaaaaaaaaaaaagaaaaaaaaaaaagcagcatattgacgctgggaaagaccagagatctgctctct

SEQ ID NO: 79 - RNA, 154 nt, synthetic construct
  source 1..154: mol_type = other RNA
aaaaaaaaaaaaaaaaaaaaaaaaaaaaaaaaaaaaaaaaaaaaaaaaagagagcagatctctgttgaataaccaacgtcaatatgctgaaaaaaaaaaaagaaaaaaaaaaaacagcatattgacgctgggaaagaccagagatctgctctct

SEQ ID NO: 80 - RNA, 155 nt, synthetic construct
  source 1..155: mol_type = other RNA
aaaaaaaaaaaaaaaaaaaaaaaaaaaaaaaaaaaaaaaaaaaaaaaaagagagcagatctctgttgaataaccaacgtcaatatgctgaaaaaaaaaaaagaaaaaaaaaaaagcagcatattgacgctgggaaagaccagagatctgctctct

SEQ ID NO: 81 - RNA, 165 nt, synthetic construct
  source 1..165: mol_type = other RNA
aaaaaaaaaaaagaaaaaaaaaaaagaaaaaaaaaaaagaaaaaaaaaaaagaaaaaaaaagagagcagatctctgttgaataaccaacgtcaatatgctgaaaaaaaaaaaagaaaaaaaaaagcagcatattgacgctgggaaagaccagagatctgctctct

SEQ ID NO: 82 - RNA, 170 nt, synthetic construct
  source 1..170: mol_type = other RNA
aaaaaaaaaaaagaaaaaaaaaaaagaaaaaaaaaaaagaaaaaaaaaaaagaaaaaaaaaaaagagagcagatctctgttgaataaccaacgtcaatatgctgaaaaaaaaaaaagaaaaaaaaaaaagcagcatattgacgctgggaaagaccagagatctgctctct

SEQ ID NO: 83 - RNA, 148 nt, synthetic construct
  source 1..148: mol_type = other RNA
aaaaaaaaaaaagaaaaaaaaaaaagaaaaaaaagagagcagatctctgttgaataaccaacgtcaatatgctgaaaaaaaaaaaagaaaaaaaaaaaagaaaaaaaacagcatattgacgctgggaaagaccagagatctgctctct

SEQ ID NO: 84 - RNA, 159 nt, synthetic construct
  source 1..159: mol_type = other RNA
aaaaaaaaaaaagaaaaaaaaaaaagaaaaaaaaaaaagagagagcagatctctgttgaataaccaacgtcaatatgctgaaaaaaaaaaaagaaaaaaaaaaaagaaaaaaaaaaaagcagcatattgacgctgggaaagaccagagatctgctctct

SEQ ID NO: 85 - RNA, 157 nt, synthetic construct
  source 1..157: mol_type = other RNA
aaaaaaaaaaaagaaaaaaaaaaaagaaaaaaaaaaaagaaaaaaaaaaaaagagagcagatctctgttgaataaccaacgtcaatatgctgaaaaaaaaaaaagaaaaaaaaaaaacagcatattgacgctgggaaagaccagagatctgctctct

SEQ ID NO: 86 - RNA, 159 nt, synthetic construct
  source 1..159: mol_type = other RNA
aaaaaaaaaaaagaaaaaaaaaaaagaaaaaaaaaaaagaaaaaaaaaaaagagagagcagatctctgttgaataaccaacgtcaatatgctgaaaaaaaaaaaagaaaaaaaaaaaagcagcatattgacgctgggaaagaccagagatctgctctct

SEQ ID NO: 87 - RNA, 220 nt, synthetic construct
  source 1..220: mol_type = other RNA
aaaaaatccaaaaaaaatctaaaaaaatcttttaaaaaaccccaaaaaaatttacaaaaaaggatccaagattaataaaaaaaaaaaaaaaaaaaaaaaaaaaaaaaagagagcagatctctgttgaataaccaacgtcaatatgctgaaaaaaaaaaaaaaaaaaaaaaaaaaaaaaaacagcatattgacgctgggaaagaccagagatctgctctct

SEQ ID NO: 88 - RNA, 288 nt, synthetic construct
  source 1..288: mol_type = other RNA
aaaaaatccaaaaaaaatctaaaaaaatcttttaaaaaaccccaaaaaaatttacaaaaaaggatccaagattaataaaaaaaaaaaaaaaaaaaaaaaaaaaaaaaagagagcagatctctgttgaataaccaacgtcaatatgctgaaaaaaaaaaaaaaaaaaaaaaaaaaaaaaaacagcatattgacgctgggaaagaccagagatctgctctctaaaaaatccaaaaaaaatctaaaaaaatcttttaaaaaaccccaaaaaaatttacaaaaaaggatcca

SEQ ID NO: 89 - RNA, 180 nt, synthetic construct
  source 1..180: mol_type = other RNA
aaaaaaaaaaaaaaaaaaaaaaaaaaaaaaaagagagcagatctctgttgaataaccaacgtcaatatgctgaaaaaatccaaaaaaaatctaaaaaaatcttttaaaaaaccccaaaaaaatttacaaaaaaggatccacagcatattgacgctgggaaagaccagagatctgctctct

SEQ ID NO: 90 - RNA, 228 nt, synthetic construct
  source 1..228: mol_type = other RNA
aaaaaaaaaaaaaaaaaaaaaaaaaaaaaaaaaaaaaaaaaaaaaaaaaaaaaaaaaaaaaaaaaaaaaaaaaaaaaaaagagagcagatctctgttgaataaccaacgtcaatatgctgaaaaaatccaaaaaaaatctaaaaaaatcttttaaaaaaccccaaaaaaatttacaaaaaaggatccacagcatattgacgctgggaaagaccagagatctgctctct

SEQ ID NO: 91 - RNA, 237 nt, synthetic construct
  source 1..237: mol_type = other RNA
aaaaaatccaaaaaaaatctaaaaaaatcttttaaaaaaccccaaaaaaatttacaaaaaaggatccaagattaataaaaaaaaaaaaaaaaaaaaaaaaaaaaaaaaaaaaaaaaaaaaaaaaagagagcagatctctgttgaataaccaacgtcaatatgctgaaaaaaaaaaaaaaaaaaaaaaaaaaaaaaaacagcatattgacgctgggaaagaccagagatctgctctct

SEQ ID NO: 92 - RNA, 215 nt, synthetic construct
  source 1..215: mol_type = other RNA
aaaaaatccaaaaaaaatctaaaaaaatcttttaaaaaaccccaaaaaaatttacaaaaaaggatccaagattaataaaaaaaaaaaaaaaaaaaaaaaaaaaaaaaaaaaaaaaaaaaaaaagagagcagatctctgttgaataaccaacgtcaatatgctgaaaaaaaaaaaacagcatattgacgctgggaaagaccagagatctgctctct

SEQ ID NO: 93 - RNA, 243 nt, synthetic construct
  source 1..243: mol_type = other RNA
aataaaaaaaaatccaaaaaaaatctaaaaaaatcttttaaaaaaccccaaaaaaatttacaaaaaaggatccaagattaataaaaaaaaaaaaaaaaaaaaaaaaaaaaaaaaaaaaaaaaaaaaaaaaagagagcagatctctgttgaataaccaacgtcaatatgctgaaaaaaaaaaaaaaaaaaaaaaaaaaaaaaaacagcatattgacgctgggaaagaccagagatctgctctct

SEQ ID NO: 94 - RNA, 221 nt, synthetic construct
  source 1..221: mol_type = other RNA
aataaaaaaaaatccaaaaaaaatctaaaaaaatcttttaaaaaaccccaaaaaaatttacaaaaaaggatccaagattaataaaaaaaaaaaaaaaaaaaaaaaaaaaaaaaaaaaaaaaaaaaaaaagagagcagatctctgttgaataaccaacgtcaatatgctgaaaaaaaaaaaacagcatattgacgctgggaaagaccagagatctgctctct

SEQ ID NO: 95 - RNA, 143 nt, synthetic construct
  source 1..143: mol_type = other RNA
aaaaaaaaaaaaaaaaaaaaaaaaaaaaaaatccggttgcgttgtgaatcgcgccactcctaacttggaccaaaaaaaaaaaaaaaaaaaaaaaaaaaaaaaaggtccaagttaggaaagtatcaactcgcaacgcaaccgga

SEQ ID NO: 96 - RNA, 144 nt, synthetic construct
  source 1..144: mol_type = other RNA
aaaaaaaaaaaaaaaaaaaaaaaaaaaaaaaagagagcagatctctgttgaataaccaacgtcaatatgctgaaaaaaaaaaaaaaaaaaaaaaaaaaaaaaaacagcatattgacttggttattcaacagagatctgctctct

SEQ ID NO: 97 - RNA, 144 nt, synthetic construct
  source 1..144: mol_type = other RNA
aaaaaaaaaaaaaaaaaaaaaaaaaaaaaaatccggttgcgttgtgaatcgcgcccacacctaacttggaccaaaaaaaaaaaaaaaaaaaaaaaaaaaaaaaaggtccaagttaggcgtgtatcaactcgcaacgcaaccgga

SEQ ID NO: 98 - RNA, 144 nt, synthetic construct
  source 1..144: mol_type = other RNA
aaaaaaaaaaaaaaaaaaaaaaaaaaaaaaatccggttgcgttgtggttgaataaccaacctaacttggaccaaaaaaaaaaaaaaaaaaaaaaaaaaaaaaaaggtccaagttaggctgggaaagacccgcaacgcaaccgga

SEQ ID NO: 99 - RNA, 144 nt, synthetic construct
  source 1..144: mol_type = other RNA
aaaaaaaaaaaaaaaaaaaaaaaaaaaaaaaccgtcgattgtccacgttgaataaccaaccggacgctagccaaaaaaaaaaaaaaaaaaaaaaaaaaaaaaaaggctagcgtccggctgggaaagaccgtggacaatcgacgg

SEQ ID NO: 100 - RNA, 118 nt, synthetic construct
  source 1..118: mol_type = other RNA
aaaaaaaaaaaaaaaaaaaaaaaaaaaaaaaagagcagatgttgaataaccaacgtctgaaaaaaaaaaaaaaaaaaaaaaaaaaaaaaaacagacgctgggaaagaccatctgctct

SEQ ID NO: 101 - RNA, 124 nt, synthetic construct
  source 1..124: mol_type = other RNA
aaaaaaaaaaaaaaaaaaaaaaaaaaaaaaaagagagcagatctgatacaacgtcaatgctgaaaaaaaaaaaaaaaaaaaaaaaaaaaaaaaacagcattgacgctggagagatctgctctct

SEQ ID NO: 102 - RNA, 117 nt, synthetic construct
  source 1..117: mol_type = other RNA
aaaaaaaaaaaaaaaaaaaaaaaaaaaaaaaagagagcagatctctgtcaatatgctgaaaaaaaaaaaaaaaaaaaaaaaaaaaaaaaacagcatattgacagagatctgctctct

SEQ ID NO: 103 - RNA, 53 nt, synthetic construct
  source 1..53: mol_type = other RNA
ggctcttctttgcctctgctggagtccggggagtggcgttggctgctagagcg

SEQ ID NO: 104 - RNA, 83 nt, synthetic construct
  source 1..83: mol_type = other RNA
ccttctttgcggctcggccattttgtcccagtcagtccggaggctgcggctgcagaagtaccgcctgcggagtaactgcaaag

SEQ ID NO: 105 - RNA, 74 nt, synthetic construct
  source 1..74: mol_type = other RNA
ccgcctcctcctgtcccgcagtcggcgtccagcggctctgcttgttcgtgtgtgtgtcgttgcaggccttattc

SEQ ID NO: 106 - RNA, 60 nt, synthetic construct
  source 1..60: mol_type = other RNA
gacctttccgagttggctgcagatttgtggtgcgttctgagccgtctgtcctgcgccaag

SEQ ID NO: 107 - RNA, 96 nt, synthetic construct
  source 1..96: mol_type = other RNA
ggaagtccgtagtgtctcattgcagataatttttagcttagggcctggtggctaggtcggttctctcctttccagtcggagacctctgccgcaaac

SEQ ID NO: 108 - RNA, 43 nt, synthetic construct
  source 1..43: mol_type = other RNA
acagttgaagaagcgaccgagggactgggagtcgttagtgagg

SEQ ID NO: 109 - RNA, 27 nt, synthetic construct
  source 1..27: mol_type = other RNA
cttcctttccaacttggacgctgcaga

SEQ ID NO: 110 - RNA, 121 nt, synthetic construct
  source 1..121: mol_type = other RNA
aagccgcagctttgaagcctgagcggccgaactcggcagctccaacccaactcggcttaactccgcctcaccgagcccagtccaagactctgtgctccctaggtttgcaacagctctctgg

SEQ ID NO: 111 - RNA, 121 nt, synthetic construct
  source 1..121: mol_type = other RNA
ggaagcattttcctgattgatgaaaaaaataactcagttatggccatctacccctgctagaaggttacagtgtattatgtagcatgcaatgtgttatgtagtgcttaataaaaataaaatg

SEQ ID NO: 112 - RNA, 70 nt, synthetic construct
  source 1..70: mol_type = other RNA
gtccacctgtccctcctgggctgctggattgtctcgttttcctgccaaataaacaggatcagcgctttac

SEQ ID NO: 113 - RNA, 190 nt, synthetic construct
  source 1..190: mol_type = other RNA
aataaggaaactgtatgaatgtctgtgggcaggaagtgaagagatccttctgtaaaggtttttggaattatgtctgctgaataataaacttttttgaaataataaatctggtagaaaaatgaaaacttgtcctcatttttctcccacactgaagaaacagggactggaacttagagtgactaaggaattt

SEQ ID NO: 114 - RNA, 57 nt, synthetic construct
  source 1..57: mol_type = other RNA
ccctgttcccagagcccacttttttttctttttttgaaataaaatagcctgtctttc

SEQ ID NO: 115 - RNA, 134 nt, synthetic construct
  source 1..134: mol_type = other RNA
actggctgcatctccctttcctctgtcctccatccttctcccaggatggtgaagggggacctggtacccagtgatccccaccccaggatcctaaatcatgacttacctgctaataaaaactcattggaaaagtg

SEQ ID NO: 116 - RNA, 90 nt, synthetic construct
  source 1..90: mol_type = other RNA
aaaaaaaaaaaaaaaaaaaaaaaaaaaaaaaaaaaaaaaaaaaaaaaaaaaaaaaaaaaaaaaaaaaaaaaaaaaaaaaaaaaaaaaaaa

SEQ ID NO: 117 - protein, 30 aa, synthetic construct
WEARLARALARALARHLARALARALRACEA

SEQ ID NO: 118 - protein, 26 aa, synthetic construct
KKALLALALHHLAHLALHLALALKKA

SEQ ID NO: 119 - protein, 26 aa, synthetic construct
KKALLAHALHLLALLALHLAHALKKA